European Patent Application EP 4 483 894 A1, published January 1, 2025. Title: PHARMACEUTICAL COMPOSITION FOR TREATING OR PREVENTING ADULT T-CELL LEUKEMIA. Applicant: NEC Corporation. Application JP. The sequence listing filed with the application follows.

SEQUENCE LISTING (81 sequences)

SEQ ID NO: 1 - protein, 9 aa, synthetic construct
  REGION 1..9: note = ATL immunogenic peptide
LLLFSAAAL

SEQ ID NO: 2 - protein, 9 aa, synthetic construct
  REGION 1..9: note = ATL immunogenic peptide
YVYDPPTTI

SEQ ID NO: 3 - protein, 9 aa, synthetic construct
  REGION 1..9: note = ATL immunogenic peptide
YTYDPPTTI

SEQ ID NO: 4 - protein, 9 aa, synthetic construct
  REGION 1..9: note = ATL immunogenic peptide
YLYDPPTTI

SEQ ID NO: 5 - protein, 9 aa, synthetic construct
  REGION 1..9: note = ATL immunogenic peptide
AQAPPTAQL

SEQ ID NO: 6 - protein, 9 aa, synthetic construct
  REGION 1..9: note = ATL immunogenic peptide
ALAPPTAQL

SEQ ID NO: 7 - protein, 9 aa, synthetic construct
  REGION 1..9: note = ATL immunogenic peptide
ALLAPAVLL

SEQ ID NO: 8 - protein, 9 aa, synthetic construct
  REGION 1..9: note = ATL immunogenic peptide
KFLEAFHEV

SEQ ID NO: 9 - protein, 9 aa, synthetic construct
  REGION 1..9: note = ATL immunogenic peptide
CLDEHQWQL

SEQ ID NO: 10 - protein, 9 aa, synthetic construct
  REGION 1..9: note = ATL immunogenic peptide
ATLAPAVLL

SEQ ID NO: 11 - protein, 9 aa, synthetic construct
  REGION 1..9: note = ATL immunogenic peptide
AALDDLRTL

SEQ ID NO: 12 - protein, 9 aa, synthetic construct
  REGION 1..9: note = ATL immunogenic peptide
ALPKIRARV

SEQ ID NO: 13 - protein, 9 aa, synthetic construct
  REGION 1..9: note = ATL immunogenic peptide
LMEEHGATL

SEQ ID NO: 14 - protein, 9 aa, synthetic construct
  REGION 1..9: note = ATL immunogenic peptide
SLVLTWAAL

SEQ ID NO: 15 - protein, 9 aa, synthetic construct
  REGION 1..9: note = ATL immunogenic peptide
VLLQQFQTA

SEQ ID NO: 16 - protein, 9 aa, synthetic construct
  REGION 1..9: note = ATL immunogenic peptide
LLITRKSFI

SEQ ID NO: 17 - protein, 9 aa, synthetic construct
  REGION 1..9: note = ATL immunogenic peptide
LMITRKSFI

SEQ ID NO: 18 - protein, 9 aa, synthetic construct
  REGION 1..9: note = ATL immunogenic peptide
ALPAPHLTL

SEQ ID NO: 19 - protein, 9 aa, synthetic construct
  REGION 1..9: note = ATL immunogenic peptide
VMSHHGEKL

SEQ ID NO: 20 - protein, 9 aa, synthetic construct
  REGION 1..9: note = ATL immunogenic peptide
IALETPVWI

SEQ ID NO: 21 - protein, 9 aa, synthetic construct
  REGION 1..9: note = ATL immunogenic peptide
IQYSSFHNL

SEQ ID NO: 22 - protein, 9 aa, synthetic construct
  REGION 1..9: note = ATL immunogenic peptide
ALQFLIPRL

SEQ ID NO: 23 - protein, 9 aa, synthetic construct
  REGION 1..9: note = ATL immunogenic peptide
LLNPNRQTI

SEQ ID NO: 24 - protein, 9 aa, synthetic construct
  REGION 1..9: note = ATL immunogenic peptide
MLPQTPSHL

SEQ ID NO: 25 - protein, 9 aa, synthetic construct
  REGION 1..9: note = ATL immunogenic peptide
ATAPPTAQL

SEQ ID NO: 26 - protein, 9 aa, synthetic construct
  REGION 1..9: note = ATL immunogenic peptide
ALRPAPALL

SEQ ID NO: 27 - protein, 9 aa, synthetic construct
  REGION 1..9: note = ATL immunogenic peptide
AVLAPAVLL

SEQ ID NO: 28 - protein, 9 aa, synthetic construct
  REGION 1..9: note = ATL immunogenic peptide
CIDEHQWQL

SEQ ID NO: 29 - protein, 9 aa, synthetic construct
  REGION 1..9: note = ATL immunogenic peptide
LIITRKSFI

SEQ ID NO: 30 - protein, 9 aa, synthetic construct
  REGION 1..9: note = ATL immunogenic peptide
LVITRKSFI

SEQ ID NO: 31 - protein, 9 aa, synthetic construct
  REGION 1..9: note = ATL immunogenic peptide
ALQPPCPNL

SEQ ID NO: 32 - protein, 9 aa, synthetic construct
  REGION 1..9: note = ATL immunogenic peptide
YQLSPPITW

SEQ ID NO: 33 - protein, 9 aa, synthetic construct
  REGION 1..9: note = ATL immunogenic peptide
TLTAWQHGL

SEQ ID NO: 34 - protein, 9 aa, synthetic construct
  REGION 1..9: note = ATL immunogenic peptide
ISAYRTCWI

SEQ ID NO: 35 - protein, 9 aa, synthetic construct
  REGION 1..9: note = ATL immunogenic peptide
FSNDFGQSL

SEQ ID NO: 36 - protein, 9 aa, synthetic construct
  REGION 1..9: note = ATL immunogenic peptide
CMIVHQGTI

SEQ ID NO: 37 - protein, 9 aa, synthetic construct
  REGION 1..9: note = ATL immunogenic peptide
SSFEFFEEA

SEQ ID NO: 38 - protein, 9 aa, synthetic construct
  REGION 1..9: note = ATL immunogenic peptide
HMAKVIEFL

SEQ ID NO: 39 - protein, 9 aa, synthetic construct
  REGION 1..9: note = ATL immunogenic peptide
CTDEHQWQL

SEQ ID NO: 40 - protein, 9 aa, synthetic construct
  REGION 1..9: note = ATL immunogenic peptide
LIEEHGATL

SEQ ID NO: 41 - protein, 9 aa, synthetic construct
  REGION 1..9: note = ATL immunogenic peptide
LLEEHGATL

SEQ ID NO: 42 - protein, 9 aa, synthetic construct
  REGION 1..9: note = ATL immunogenic peptide
LTEEHGATL

SEQ ID NO: 43 - protein, 9 aa, synthetic construct
  REGION 1..9: note = ATL immunogenic peptide
LVEEHGATL

SEQ ID NO: 44 - protein, 9 aa, synthetic construct
  REGION 1..9: note = ATL immunogenic peptide
YFFTVIFSF

SEQ ID NO: 45 - protein, 9 aa, synthetic construct
  REGION 1..9: note = ATL immunogenic peptide
LTITRKSFI

SEQ ID NO: 46 - protein, 9 aa, synthetic construct
  REGION 1..9: note = ATL immunogenic peptide
LAITRKSFI

SEQ ID NO: 47 - protein, 9 aa, synthetic construct
  REGION 1..9: note = ATL immunogenic peptide
EAIDGYITL

SEQ ID NO: 48 - protein, 9 aa, synthetic construct
  REGION 1..9: note = ATL immunogenic peptide
TVLVPPRNL

SEQ ID NO: 49 - protein, 9 aa, synthetic construct
  REGION 1..9: note = ATL immunogenic peptide
AYRTCWIFS

SEQ ID NO: 50 - protein, 9 aa, synthetic construct
  REGION 1..9: note = ATL immunogenic peptide
AQISAYRTC

SEQ ID NO: 51 - protein, 9 aa, synthetic construct
  REGION 1..9: note = ATL immunogenic peptide
GTHLDAGTV

SEQ ID NO: 52 - protein, 9 aa, synthetic construct
  REGION 1..9: note = ATL immunogenic peptide
YPGWHSTTI

SEQ ID NO: 53 - protein, 9 aa, synthetic construct
  REGION 1..9: note = ATL immunogenic peptide
ETLQFIDSM

SEQ ID NO: 54 - protein, 9 aa, synthetic construct
  REGION 1..9: note = ATL immunogenic peptide
VLPPARHST

SEQ ID NO: 55 - protein, 9 aa, synthetic construct
  REGION 1..9: note = ATL immunogenic peptide
SSLDPPKVL

SEQ ID NO: 56 - protein, 9 aa, synthetic construct
  REGION 1..9: note = ATL immunogenic peptide
SLPFSPSQF

SEQ ID NO: 57 - protein, 9 aa, synthetic construct
  REGION 1..9: note = ATL immunogenic peptide
FIDSDSSSW

SEQ ID NO: 58 - protein, 9 aa, synthetic construct
  REGION 1..9: note = ATL immunogenic peptide
CDLSSFEFF

SEQ ID NO: 59 - protein, 9 aa, synthetic construct
  REGION 1..9: note = ATL immunogenic peptide
ATGDCSSFI

SEQ ID NO: 60 - protein, 9 aa, synthetic construct
  REGION 1..9: note = ATL immunogenic peptide
LPFSPSQFL

SEQ ID NO: 61 - protein, 9 aa, synthetic construct
  REGION 1..9: note = ATL immunogenic peptide
LAEEHGATL

SEQ ID NO: 62 - protein, 9 aa, synthetic construct
  REGION 1..9: note = ATL immunogenic peptide
SLLITRKSF

SEQ ID NO: 63 - protein, 9 aa, synthetic construct
  REGION 1..9: note = ATL immunogenic peptide
LHITRKSFI

SEQ ID NO: 64 - protein, 9 aa, synthetic construct
  REGION 1..9: note = ATL immunogenic peptide
HMTSSERPF

SEQ ID NO: 65 - protein, 9 aa, synthetic construct
  REGION 1..9: note = ATL immunogenic peptide
GYITCERPF

SEQ ID NO: 66 - protein, 9 aa, synthetic construct
  REGION 1..9: note = ATL immunogenic peptide
VFGRVMQID

SEQ ID NO: 67 - protein, 9 aa, synthetic construct
  REGION 1..9: note = ATL immunogenic peptide
VMQIDGVQP

SEQ ID NO: 68 - protein, 9 aa, synthetic construct
  REGION 1..9: note = ATL immunogenic peptide
GRVMQIDGV

SEQ ID NO: 69 - protein, 9 aa, synthetic construct
  REGION 1..9: note = ATL immunogenic peptide
SLPNEKQTS

SEQ ID NO: 70 - protein, 9 aa, synthetic construct
  REGION 1..9: note = ATL immunogenic peptide
ILSDHQQSQ

SEQ ID NO: 71 - protein, 9 aa, synthetic construct
  REGION 1..9: note = ATL immunogenic peptide
STGESAQTS

SEQ ID NO: 72 - protein, 9 aa, synthetic construct
  REGION 1..9: note = ATL immunogenic peptide
GSPDEFSND

SEQ ID NO: 73 - protein, 9 aa, synthetic construct
  REGION 1..9: note = ATL immunogenic peptide
SPDEFSNDF

SEQ ID NO: 74 - protein, 9 aa, synthetic construct
  REGION 1..9: note = ATL immunogenic peptide
GILSDHQQS

SEQ ID NO: 75 - protein, 9 aa, synthetic construct
  REGION 1..9: note = ATL immunogenic peptide
THLDAGTVE

SEQ ID NO: 76 - protein, 9 aa, synthetic construct
  REGION 1..9: note = ATL immunogenic peptide
LPPARHSTI

SEQ ID NO: 77 - protein, 9 aa, synthetic construct
  REGION 1..9: note = ATL immunogenic peptide
ARHSTIPLV

SEQ ID NO: 78 - protein, 9 aa, synthetic construct
  REGION 1..9: note = ATL immunogenic peptide
IFADVSSST

SEQ ID NO: 79 - protein, 9 aa, synthetic construct
  REGION 1..9: note = ATL immunogenic peptide
LHEEHGATL

SEQ ID NO: 80 - protein, 9 aa, synthetic construct
  REGION 1..9: note = ATL immunogenic peptide
GYITLGKPH

SEQ ID NO: 81 - protein, 9 aa, synthetic construct
  REGION 1..9: note = ATL immunogenic peptide
ASPSHMTSM